European Patent Specification EP 3 412 776 B1, published April 10, 2024. Title: GENETIC POLYMORPHISM ASSOCIATED WITH DOG AFIBRINOGENEMIA. Applicant: Stiftung Tieraerztliche Hochschule Hannover. Application not yet assigned. The sequence listing filed with the application follows.

SEQUENCE LISTING (8 sequences)

SEQ ID NO: 1 - DNA, 8914 bp, Canis familiaris
  gDNA fibrinogen alpha chain (FGA) gene: FGA:g.6296T/delT, NCBI Reference Sequence: NC_006597.3, >gi|357579616:c52246989-52238076 Canis lupus familiaris breed boxer chromosome 15, CanFam3.1, whole genome shotgun sequence
agagtggaggcagtcttcctttctttcagctggagtgctcctcaagagcgagctccacccttaaaaaagatgttttctgcgaagatcttgtgcctggtcctgagtgtggtgggcacagtctgggtatggccgcctttactttctcttcttgctttctctctggtgttcattctgcaaaacgcttgcaggtctgagtcagtcttaagtttgtccttgcacactgttgactttataagctctaggccatggaggcaagttcctagatgagtctgacacctcaggagtaagagggagacttaactggaccaatgaatagaaattcacaggggaagctttggtatctgtaattcagccttacaacattgtttatttgttttgagggaagaaatctttgccatctttgttccaataaagccttgggatagttcatgctagctaacagaaaaaaaagcattcttctgatgagaattttaaaaatctaatgattaatttattgctagttgtccataataagcagaacagtggtttaatgtagttttctgaaaggttgtttgtgggtgtgggtgtgtgtttttaaagaaaagcaaattagttgtctttgaaaacatctaaaacaatattttattacatattacatagtcgggagacattaattgagaaggcaatatcctttttgtgggaaggaatcttttaaaataattactaaatattgctataatttctaaagtttgactccagagacctatagaagagaaacctcattcaagatgctttcgaaacccttagatcttataaaaacatgataaatatgtttaagaaactcaattactttcaggatatgaattattccaatttttttctttcccttcaccactcataaatcctactatcagagcaaaagaactaaagaggttttctaacctaatattcttccttatagtaaactaataagtaaaaaatttggaagactaacatcatttactaacatgatatgttggatatctctcccttattgacataagtattgaattttgcctatttttattgttgtgccattttattctgaagtatgtttgaatttataattttatttcttaaagatattgtacttgttcctttaaataaactgtccttaattgctgatttatttattattattatttttattgttaggatactttaaaaaaatgagacagcaaatattaggtaattataagaataaactaaaaaaaattataagaataaactattcaagggagtacctggttagctcagtcggtagaggatgtgactcttgatctctgggttgtgagtttgagtccctactgggcatagagagtacttaaaaacaaacaaacaaaaagaataaactatccgagattaaaatagtcatagcaaaaatccttggtatgttagtgatacaaaataaaaatagctaaaacgtaaaacttatcttgatttattaggatgtaaagtctaattggaagatttttatgtcctatttcacttcataggtcacaatagaaatttttttaaaaatctgtatttctgaatagagggtgctcaaaaaaagttgtcagtccattatttttctttcagtctactcttttgcattgcaaaaggaaattattaaaatttcctttataattcctttatattaaaggaatattaaaatattaaaattcttttataattaaaattataattattaaaattataaaaggacattattacatgagcgggtaacctcaaaagcattttccagtccttattggccacatttgtatccttggtatgttcttgctcaaattacggacccataagaccgaagtagaaacttgaagtagagagaaattaaactaaggtagtataggtttggtcctactaaaacagaaattataggagaaagaactctgaattttccaaatacccttccatctccagacattactgaaaatgaaaaggtaaattttaattacttttgttgattcaaatattttctcttctataataaatcctttaagacacctagcttcattaaatgcttgtttcgtgtccaacacagttaaaaaatgtctataccctgtctccttcaattcataaaactccatgaagtaggtatttggattttcaatcaaaatgtaagaaaaatgaagcttgcagaggccccagagctgctgctcttaatctctgggagaaccctcccctccttgggatttacaggcttgacagtgtcttctccttatctgcctaatgctgttctctttcgtgtgtatgaatgaatccgtaaagaccacaaattccaaagaaggtgaatttatagccgaaggaggaggtgtacgtggcccaagaattgtggaaagacagcaatctgcctgcaaggagacagactggcccttctgttccgatgaagactgggtgagcaatgggcatagggagggggataatcctcccctgtggtgctagaattgtgcacaaactgacccagaaagtcacagaaaacttttccaacgggtaataatctaataactcattacatgccaaattaaaaaagacaattggaaagtagcctcaccatgagagcactatttaaattacctcccaaaccctgggtcattagtgggattgatagcttggattttagttgcatgttccagcaaatgccaggaacctgagtattatggcttcaagattttgtggagcctaatttatggttaagtggaccttcattccagaatttctctatgactagttctctcaaaccacttttaagtcaatagatgatcagaggatgttgggggagggcaatgggagccacatggaaacttttaaaattgtactggattcaaatagaggctttaatataattttccccttcccttccagaactacaaatgcccttctggctgcaggatgaaagggttaatcgatgaagtcaatcaagattttacaaacagaataaataagctcaaaaactcactctttgactatcagaagaacaataaggactctagttcattgacaacgaatataatggaacttgtgagaggggattttgccactgccaacagtaagtagtaacatctgggctttgactttatagcgcacaacagagaaacaaccaaggccctaaataaatacactgtctccttatggcaacttccaattgtattccaaagtacttaagatagaaacacatgccttcacgataccctgaattttaaggaggggcttgctttttgtaaaaggaacattaaaaaggtcagtttagaattaaaaacagtcagtttagaattgtttaaagtcatggaacacctgggtggctcagaggttgagcatctgcctttggttcagggtgtgatctcagggtcctgagatcgagttccacatcgggctccccgcagggagcctgcttctccctctgcctgtgtctctgcctctctctctctctgtctcccaggaataaataatctttttttaaaaaaaattgtttcaagtcacaaaattaagtctgaactttgtattgaagactagaatttatgtgtgttcttttttaagagtatatactgaaaataagatgagcaaagccttttgagtagatcttgtttctgtcttatagaggatggagaaaactgagagatcaagggacttattcgaagacacaaagctatcatgtgatgaggctgggagttcagtttacaaactccatcaggctgttcatgttttgtttttttcaatttaagatatagaatcatgctctgtattcctcacagaactatgactaagtctcattaggactaggaaacactggatttgctcttggaatgggaagcaagtttagtgatggcctagctccagaagctttgactctttatacctttaggggacacttgactaatttaaaatcaacaatgcaacagcaatggcaggagagtgatcctattgacctgaaaaaagaaaatctcaggaacaatttcagatctataggtaggagggaaaactcagaaaatccaagacgatgtttaagtatgttatcatattatttagcaatatgtttaaggatatgatggttaaggttaaggatatgatgaaatagttgaaatgcaatcacatttaatctcctaattatacctttaaaattccaaagaaatttcttccgcatttatttgggttactaattgctagtagacaatcttaactgacgctatggatgactaaagaatataacattgtccaaacatcaaatgcctattagattgggaactaacaaataaagtgtccagagaacaaattgttattaaaagggaaaggatatttatgaacaaatttccttcttttgctagctattataagcaaatcacttagctgttccttcactatccatactcctttttttttttccagataatgataatacatatagccaagtgtcagaagatctgagaagcaaaattgagatcctgaggcgcaaagtcctagaacaagtacaacacatccaccttctacagaaaaatgtcagggatcagctggtagatatgaaacgactagaggtaagcaagtatgtggctgtgacatcagatttccttgtctttgaacagcagggtaaaggaaggcgatagtcattcaccgaaggcctactgtatgtagagcaaagtgttacatccattatgcacctacaaagcaggtattatttcccccactctacagatgaagaaaaaaaagctcagtgatataagtaaattttccaaggatacacagttagtacatttctaaaggaaatattaggtccccgcttgtcttgttccaaagccctgacaaggccatgcctctggacctctagtcgtagtctcactaaggatcaattcatcagtgcttcctttcagagggaatagcatcttactcttgatctattttaaggctaagatgaatccaaatagctcctattgcttatctggcctaactttacaaaacctaatgtctcttccactgagggcatgacatacatgaaaaataagagtattgattggtaggtctccaagtcagagaaatgaacccagttcagttctgctaagaacttaataagcatatattttttaatttatatcaacctcttttctatacctttctccccttctctctaggtggacattgatattaagatccgatcttgccaagggtcatgcagtagggctttagagcgtaggacagatctaaagtactatgaagatcaacagaagcaacttgaacaagtcattgccaaagacttacttccacctaaagacaggcaatacttaccactgctaaaaacgagcccagctccaaatatgcttcctggggactacaagagccagcttcaggaggcccctctggagtggaaggcactcatggaaatgaagcagatgaaaatgactctagagaggcttgatagagatgggaatgcccgaggagacactccatctcatggaacaggatcagtgcctgaaagccccaggaaccctgggagctccacccctggaagtgctggcacttggaaccctggcagcactggacctggcagtgctggtccttggagctctgggagcaccaggcctggcagcactgggcctggtagtgctggtacttggagcaccaggcctggcagcactgggcctggcagtgctggtacttggagctccgggagcaccgggcctggcagcactggaccaggcagtaccggtacttggagctctgggagcaccgggcctggcagcactggaccaggcagtaccggtacttggagctccgggagcaccgggcctggcaacactggactgggcagtactggcacttggagctccgggagcaccgggcctggcaacactggaccgggcagtactggcacttggagctctggaagttctgactccgaaagctttaggccaggtagcgtagggcatgggaacaccaggcctaccaacccagagtgggggacatttgaagaggtgtcaggaagtgtgactccagggttaaagaatgagttccacacaggtaaactggtcacttctaaaggagagaaagagcttcttattggtaatgagaaggtcacctctggtagcacaaccaccactcgtcacgcatgctctaaaactgttactaagaccgttataggtccagatggtcgcaaagaagtgacaaaagaagtggtaaactccgaagatggttctgattgtggtgacttatcccatacttttgctggcagcctagatgatctccatgctaggcaccctgatctagagcgtttctttggcacctcaattgtcaaaacacctccaggtatacttttaccctcgcgtaaagagtttgaacataagacccacattatgggctcagattctgacatattcacaaacatagggacacctgagttcccttccagtggtaaaacttcaagtcacagcaaacaatttgtgaccagtagtacgacttacaacagaggagactccgcatttgaaagcaagagctataaaggggcaggtgaggccggaacggaagcagaacgtgaaatcttcagaggagaatatagcatcaaaagaggccatgctaaagctcgccctgccagaggtatccgcacttctcctttggggaagccttccctgaccccctagactaagttctctattcttgcaatgcctcccatggcaccttgaacctctttcctagccctctatgacactttatagaaattacaccttttgtttgtttgtgtttggggactagactgtaagttccatgagggcaagggttttgtctatcatgtgtattcctaaatgcccaacagtgcagagagtcatcactcaataaatgcatgtcaaatgaatgaatgaatccctccgaaattccatttcaagtttgtctaaccaaattctttcgctattcaaaatgtgtgctcttgcaactgtcacccaattcattaatcgtatttttagtgtgtgtctcagttgacattgagatcaggttaaaaacaagttatattacaaccaaatgatgcctagatatctttggtggttacttgctgttatcagtaccggcaagtaaaatttcaaatccattggagaaaatcccctttgcaatttataggtataaatgtcactcacttgcatgagtttcatcccagtgtaagtgtgtcctttccccatggagagaaggaaggaaggaaggaaggaaggaaggaaggaaggaaggaaggaaggaaaagaaagccagtatcttcctgtcttcatttaatctgggccatgcctatctttgtaaagttaaatgagaataagttcttccaaccagcttaattttttttttagactgtgatgatgtcctccaaacacatccttcaggtgcccaaagtggtattttcaatatcaagctaccgggatccagtaagcttttttctgtttattgtgatcaagagaccagtctgggaggatggcttttgatccagcagagaatggatggatcactgaattttaaccggacctggcaagactacaagagaggtttcggcagcctggatgacaagggggaaggcgagttctggctaggcaatgaacacctccacttactaaccctgagggcctctgtccttcgggttgaattagaggactgggctgggaaccaggcttatgcggaatatcacctgagggtaggctctgaggcagagggctatgccctgcaggtctcctcctacgagggcacagcaggggatgctctggtggagggttctgcagaggaaggaacagagtatacctctcacgcgggcatgcagttcagcacgtacgacagggatgcagaccagtgggaagagaactgtgcagaagtctacggaggaggctggtggtacaacagctgccaagcggccaatctcaatggcatctactaccctgggggctcctatgatccaaggaacaacagtccttatgagattgaaaatggagtggtctgggtccccttcagaggtgcagattattccctcagggctgttcgcatgaaaatcaggcccctggagaccaggtaggagtggaagtgagagtaatctgttttctttgtttagggaggtgaagaagaaaaaaaaaatggggaagataaagtagttaagattctttacaatccactaaaaaaattcacaggtgctattttattatttcttgtactgtatctaaatgtaactgagacatattactgctttaaagaataaagttatgtgagcttttttatcttgaaaggaactctgggttttcaagtttctctaaggatacaccaaggaacatcaggaagaagaaactcatggatgctcctctctttaacccttaagggtgttcttttgagccctcctctcctcacaccactcgaagtcatagggccactgtaaagaaaaaagttattgcatccattttgtttaaatgggttgaaaccaatattttaagtgacaaatcactgaattgaacaatagctggccttggtagagggacttagagactacgaaatacatccatcacttctgttagcaagcaagtccaggaaggcaggagaagcattctttcctaatagaaacagagatctattctttatgcttttcgtgaagaccataatgcacatttaattttttccccagaggctaacaagtctctttcagaaacacatggcatgaaaaaaaaatgcatttaaaatcctttaaacgtttataagtattcaaaaaccactactactgttaatgaattcataaattcagtgtatttacactggtcagtattttatttgatgtatgttgcatttttgatcttggcagccttggctcctgccccctcattttaaacttatattctttctagaggactacttgccatttgcatttgaaaatgtattaaaatactccaagcacactggg

SEQ ID NO: 2 - DNA, 3618 bp, Canis familiaris
  mRNA fibrinogen alpha chain (FGA) gene: FGA:g.1734T/delT, NCBI Reference Sequence: XM_532697.5, >XM_532697.5, Predicted: Canis lupus familiaris fibrinogen alpha chain (FGA), mRNA
agagtggaggcagtcttcctttctttcagctggagtgctcctcaagagcgagctccacccttaaaaaagatgttttctgcgaagatcttgtgcctggtcctgagtgtggtgggcacagtctggaccacaaattccaaagaaggtgaatttatagccgaaggaggaggtgtacgtggcccaagaattgtggaaagacagcaatctgcctgcaaggagacagactggcccttctgttccgatgaagactggaactacaaatgcccttctggctgcaggatgaaagggttaatcgatgaagtcaatcaagattttacaaacagaataaataagctcaaaaactcactctttgactatcagaagaacaataaggactctagttcattgacaacgaatataatggaacttgtgagaggggattttgccactgccaacaataatgataatacatatagccaagtgtcagaagatctgagaagcaaaattgagatcctgaggcgcaaagtcctagaacaagtacaacacatccaccttctacagaaaaatgtcagggatcagctggtagatatgaaacgactagaggtggacattgatattaagatccgatcttgccaagggtcatgcagtagggctttagagcgtaggacagatctaaagtactatgaagatcaacagaagcaacttgaacaagtcattgccaaagacttacttccacctaaagacaggcaatacttaccactgctaaaaacgagcccagctccaaatatgcttcctggggactacaagagccagcttcaggaggcccctctggagtggaaggcactcatggaaatgaagcagatgaaaatgactctagagaggcttgatagagatgggaatgcccgaggagacactccatctcatggaacaggatcagtgcctgaaagccccaggaaccctgggagctccacccctggaagtgctggcacttggaaccctggcagcactggacctggcagtgctggtccttggagctctgggagcaccaggcctggcagcactgggcctggtagtgctggtacttggagcaccaggcctggcagcactgggcctggcagtgctggtacttggagctccgggagcaccgggcctggcagcactggaccaggcagtaccggtacttggagctctgggagcaccgggcctggcagcactggaccaggcagtaccggtacttggagctccgggagcaccgggcctggcaacactggactgggcagtactggcacttggagctccgggagcaccgggcctggcaacactggaccgggcagtactggcacttggagctctggaagttctgactccgaaagctttaggccaggtagcgtagggcatgggaacaccaggcctaccaacccagagtgggggacatttgaagaggtgtcaggaagtgtgactccagggttaaagaatgagttccacacaggtaaactggtcacttctaaaggagagaaagagcttcttattggtaatgagaaggtcacctctggtagcacaaccaccactcgtcacgcatgctctaaaactgttactaagaccgttataggtccagatggtcgcaaagaagtgacaaaagaagtggtaaactccgaagatggttctgattgtggtgacttatcccatacttttgctggcagcctagatgatctccatgctaggcaccctgatctagagcgtttctttggcacctcaattgtcaaaacacctccaggtatacttttaccctcgcgtaaagagtttgaacataagacccacattatgggctcagattctgacatattcacaaacatagggacacctgagttcccttccagtggtaaaacttcaagtcacagcaaacaatttgtgaccagtagtacgacttacaacagaggagactccgcatttgaaagcaagagctataaaggggcaggtgaggccggaacggaagcagaacgtgaaatcttcagaggagaatatagcatcaaaagaggccatgctaaagctcgccctgccagagactgtgatgatgtcctccaaacacatccttcaggtgcccaaagtggtattttcaatatcaagctaccgggatccagtaagcttttttctgtttattgtgatcaagagaccagtctgggaggatggcttttgatccagcagagaatggatggatcactgaattttaaccggacctggcaagactacaagagaggtttcggcagcctggatgacaagggggaaggcgagttctggctaggcaatgaacacctccacttactaaccctgagggcctctgtccttcgggttgaattagaggactgggctgggaaccaggcttatgcggaatatcacctgagggtaggctctgaggcagagggctatgccctgcaggtctcctcctacgagggcacagcaggggatgctctggtggagggttctgcagaggaaggaacagagtatacctctcacgcgggcatgcagttcagcacgtacgacagggatgcagaccagtgggaagagaactgtgcagaagtctacggaggaggctggtggtacaacagctgccaagcggccaatctcaatggcatctactaccctgggggctcctatgatccaaggaacaacagtccttatgagattgaaaatggagtggtctgggtccccttcagaggtgcagattattccctcagggctgttcgcatgaaaatcaggcccctggagaccaggtaggagtggaagtgagagtaatctgttttctttgtttagggaggtgaagaagaaaaaaaaaatggggaagataaagtagttaagattctttacaatccactaaaaaaattcacaggtgctattttattatttcttgtactgtatctaaatgtaactgagacatattactgctttaaagaataaagttatgtgagcttttttatcttgaaaggaactctgggttttcaagtttctctaaggatacaccaaggaacatcaggaagaagaaactcatggatgctcctctctttaacccttaagggtgttcttttgagccctcctctcctcacaccactcgaagtcatagggccactgtaaagaaaaaagttattgcatccattttgtttaaatgggttgaaaccaatattttaagtgacaaatcactgaattgaacaatagctggccttggtagagggacttagagactacgaaatacatccatcacttctgttagcaagcaagtccaggaaggcaggagaagcattctttcctaatagaaacagagatctattctttatgcttttcgtgaagaccataatgcacatttaattttttccccagaggctaacaagtctctttcagaaacacatggcatgaaaaaaaaatgcatttaaaatcctttaaacgtttataagtattcaaaaaccactactactgttaatgaattcataaattcagtgtatttacactggtcagtattttatttgatgtatgttgcatttttgatcttggcagccttggctcctgccccctcattttaaacttatattctttctagaggactacttgccatttgcatttgaaaatgtattaaaatactccaagcacactggg

SEQ ID NO: 3 - protein, 586 aa, Canis familiaris
  Transcript FGA202 (ENSCAFT00000013402.2), affected dog
MFSAKILCLVLSVVGTVWTTNSKEGEFIAEGGGVRGPRIVERQQSACKETDWPFCSDEDWNYKCPSGCRMKGLIDEVNQDFTNRINKLKNSLFDYQKNNKDSSSLTTNIMELVRGDFATANNNDNTYSQVSEDLRSKIEILRRKVLEQVQHIHLLQKNVRDQLVDMKRLEVDIDIKIRSCQGSCSRALERRTDLKYYEDQQKQLEQVIAKDLLPPKDRQYLPLLKTSPAPNMLPGDYKSQLQEAPLEWKALMEMKQMKMTLERLDRDGNARGDTPSHGTGSVPESPRNPGSSTPGSAGTWNPGSTGPGSAGPWSSGSTRPGSTGPGSAGTWSTRPGSTGPGSAGTWSSGSTGPGSTGPGSTGTWSSGSTGPGSTGPGSTGTWSSGSTGPGNTGLGSTGTWSSGSTGPGNTGPGSTGTWSSGSSDSESFRPGSVGHGNTRPTNPEWGTFEEVSGSVTPGLKNEFHTGKLVTSKGEKELLIGNEKVTSGSTTTTRHACSKTVTKTVIGPDGRKEVTKEVVNSEDGSDCGDLSHTFAGSLDDLHARHPDLERFFGTSMSKHLQVYFYPRVKSLNIRPTLWAQILTYSQT

SEQ ID NO: 4 - protein, 892 aa, Canis familiaris
  Transcript FGA202 (ENSCAFT00000013402.2), unaffected dog
MFSAKILCLVLSVVGTVWTTNSKEGEFIAEGGGVRGPRIVERQQSACKETDWPFCSDEDWNYKCPSGCRMKGLIDEVNQDFTNRINKLKNSLFDYQKNNKDSSSLTTNIMELVRGDFATANNNDNTYSQVSEDLRSKIEILRRKVLEQVQHIHLLQKNVRDQLVDMKRLEVDIDIKIRSCQGSCSRALERRTDLKYYEDQQKQLEQVIAKDLLPPKDRQYLPLLKTSPAPNMLPGDYKSQLQEAPLEWKALMEMKQMKMTLERLDRDGNARGDTPSHGTGSVPESPRNPGSSTPGSAGTWNPGSTGPGSAGPWSSGSTRPGSTGPGSAGTWSTRPGSTGPGSAGTWSSGSTGPGSTGPGSTGTWSSGSTGPGSTGPGSTGTWSSGSTGPGNTGLGSTGTWSSGSTGPGNTGPGSTGTWSSGSSDSESFRPGSVGHGNTRPTNPEWGTFEEVSGSVTPGLKNEFHTGKLVTSKGEKELLIGNEKVTSGSTTTTRHACSKTVTKTVIGPDGRKEVTKEVVNSEDGSDCGDLSHTFAGSLDDLHARHPDLERFFGTSIVKTPPGILLPSRKEFEHKTHIMGSDSDIFTNIGTPEFPSSGKTSSHSKQFVTSSTTYNRGDSAFESKSYKGAGEAGTEAEREIFRGEYSIKRGHAKARPARDCDDVLQTHPSGAQSGIFNIKLPGSSKLFSVYCDQETSLGGWLLIQQRMDGSLNFNRTWQDYKRGFGSLDDKGEGEFWLGNEHLHLLTLRASVLRVELEDWAGNQAYAEYHLRVGSEAEGYALQVSSYEGTAGDALVEGSAEEGTEYTSHAGMQFSTYDRDADQWEENCAEVYGGGWWYNSCQAANLNGIYYPGGSYDPRNNSPYEIENGVVWVPFRGADYSLRAVRMKIRPLETR

SEQ ID NO: 5 - protein, 517 aa, Canis familiaris
  Transcript FGA201 (ENSCAFT00000043702.2), affected dog
MKGLIDEVNQDFTNRINKLKNSLFDYQKNNKDSSSLTTNIMELVRGDFATANNNDNTYSQVSEDLRSKIEILRRKVLEQVQHIHLLQKNVRDQLVDMKRLEVDIDIKIRSCQGSCSRALERRTDLKYYEDQQKQLEQVIAKDLLPPKDRQYLPLLKTSPAPNMLPGDYKSQLQEAPLEWKALMEMKQMKMTLERLDRDGNARGDTPSHGTGSVPESPRNPGSSTPGSAGTWNPGSTGPGSAGPWSSGSTRPGSTGPGSAGTWSTRPGSTGPGSAGTWSSGSTGPGSTGPGSTGTWSSGSTGPGSTGPGSTGTWSSGSTGPGNTGLGSTGTWSSGSTGPGNTGPGSTGTWSSGSSDSESFRPGSVGHGNTRPTNPEWGTFEEVSGSVTPGLKNEFHTGKLVTSKGEKELLIGNEKVTSGSTTTTRHACSKTVTKTVIGPDGRKEVTKEVVNSEDGSDCGDLSHTFAGSLDDLHARHPDLERFFGTSMSKHLQVYFYPRVKSLNIRPTLWAQILTYSQT

SEQ ID NO: 6 - protein, 823 aa, Canis familiaris
  Transcript FGA201 (ENSCAFT00000043702.2), unaffected dog
MKGLIDEVNQDFTNRINKLKNSLFDYQKNNKDSSSLTTNIMELVRGDFATANNNDNTYSQVSEDLRSKIEILRRKVLEQVQHIHLLQKNVRDQLVDMKRLEVDIDIKIRSCQGSCSRALERRTDLKYYEDQQKQLEQVIAKDLLPPKDRQYLPLLKTSPAPNMLPGDYKSQLQEAPLEWKALMEMKQMKMTLERLDRDGNARGDTPSHGTGSVPESPRNPGSSTPGSAGTWNPGSTGPGSAGPWSSGSTRPGSTGPGSAGTWSTRPGSTGPGSAGTWSSGSTGPGSTGPGSTGTWSSGSTGPGSTGPGSTGTWSSGSTGPGNTGLGSTGTWSSGSTGPGNTGPGSTGTWSSGSSDSESFRPGSVGHGNTRPTNPEWGTFEEVSGSVTPGLKNEFHTGKLVTSKGEKELLIGNEKVTSGSTTTTRHACSKTVTKTVIGPDGRKEVTKEVVNSEDGSDCGDLSHTFAGSLDDLHARHPDLERFFGTSIVKTPPGILLPSRKEFEHKTHIMGSDSDIFTNIGTPEFPSSGKTSSHSKQFVTSSTTYNRGDSAFESKSYKGAGEAGTEAEREIFRGEYSIKRGHAKARPARDCDDVLQTHPSGAQSGIFNIKLPGSSKLFSVYCDQETSLGGWLLIQQRMDGSLNFNRTWQDYKRGFGSLDDKGEGEFWLGNEHLHLLTLRASVLRVELEDWAGNQAYAEYHLRVGSEAEGYALQVSSYEGTAGDALVEGSAEEGTEYTSHAGMQFSTYDRDADQWEENCAEVYGGGWWYNSCQAANLNGIYYPGGSYDPRNNSPYEIENGVVWVPFRGADYSLRAVRMKIRPLETR

SEQ ID NO: 7 - DNA, 20 bp, Artificial Sequence
  Primer
ttggagctctggaagttctg

SEQ ID NO: 8 - DNA, 20 bp, Artificial Sequence
  Primer
ctttagcatggcctcttttg